European Patent Specification EP 3 923 984 B1, published May 20, 2026. Title: A method of treatment and prophylaxis. Applicant: Hudson Institute of Medical Research. The sequence listing filed with the application follows.

SEQUENCE LISTING (19 sequences)

SEQ ID NO: 1 - protein, 28 aa, Homo sapiens
GFGGGYGGGLGAGLGGGFGGGFAGGDGL

SEQ ID NO: 2 - DNA, 354 bp, Mus musculus
caggtgcagctgaaggagtcaggacctggcctggtggcaccctcacagagcctgtccatcacatgcactgtctctgggttctcattatccagatatagtgtacactgggttcgccagcctccaggaaagggtctggagtggctgggaatgatatggggtggtggaagcacagactataattcagctctcaaatccagactgagcatcagcaaggacaactccaagagccaagttttcttaaaaatgaacagtctgcaaactgatgacacagccatgtactactgtgccagaaaagactacggctactcctactttgactactggggccaaggcaccactctcacagtctcctca

SEQ ID NO: 3 - protein, 118 aa, Mus musculus
QVQLKESGPGLVAPSQSLSITCTVSGFSLSRYSVHWVRQPPGKGLEWLGMIWGGGSTDYNSALKSRLSISKDNSKSQVFLKMNSLQTDDTAMYYCARKDYGYSYFDYWGQGTTLTVSS

SEQ ID NO: 4 - DNA, 363 bp, Mus musculus
gatgttttgatgacccaaactccactctccctgcctgtcagtcttggagatcaagcctccatctcttgcagatctagtcagagcattgtacatagtaatggaaacacctatttagaatggtacctgcagaaaccaggccagtctccaaagctcctgatctacaaagtttccaaccgattttctggggtcccagacaggttcagtggcagtggatcagggacagatttcacactcaagatcagcagagtggaggctgaggatctgggagtttattactgctttcaaggttcacatgttccattcacgttcggctcggggacaaagttggaaataaaacgggctgatgctgcaccaactgtatcc

SEQ ID NO: 5 - protein, 121 aa, Mus musculus
DVLMTQTPLSLPVSLGDQASISCRSSQSIVHSNGNTYLEWYLQKPGQSPKLLIYKVSNRFSGVPDRFSGSGSGTDFTLKISRVEAEDLGVYYCFQGSHVPFTFGSGTKLEIKRADAAPTVS

SEQ ID NO: 6 - protein, 8 aa, Mus musculus
GFSLSRYS

SEQ ID NO: 7 - protein, 7 aa, Mus musculus
IWGGGST

SEQ ID NO: 8 - protein, 12 aa, Mus musculus
ARKDYGYSYFDY

SEQ ID NO: 9 - protein, 11 aa, Mus musculus
QSIVHSNGNTY

SEQ ID NO: 10 - protein, 3 aa, Mus musculus
KVS

SEQ ID NO: 11 - protein, 9 aa, Mus musculus
FQGSHVPFT

SEQ ID NO: 12 - protein, 25 aa, Mus musculus
QVQLKESGPGLVAPSQSLSITCTVS

SEQ ID NO: 13 - protein, 17 aa, Mus musculus
VHWVRQPPGKGLEWLGM

SEQ ID NO: 14 - protein, 38 aa, Mus musculus
DYNSALKSRLSISKDNSKSQVFLKMNSLQTDDTAMYYC

SEQ ID NO: 15 - protein, 11 aa, Mus musculus
WGQGTTLTVSS

SEQ ID NO: 16 - protein, 26 aa, Mus musculus
DVLMTQTPLSLPVSLGDQASISCRSS

SEQ ID NO: 17 - protein, 17 aa, Mus musculus
LEWYLQKPGQSPKLLIY

SEQ ID NO: 18 - protein, 36 aa, Mus musculus
NRFSGVPDRFSGSGSGTDFTLKISRVEAEDLGVYYC

SEQ ID NO: 19 - protein, 19 aa, Mus musculus
FGSGTKLEIKRADAAPTVS